European Patent Application EP 4 711 447 A1, published March 18, 2026. Title: 신경근 오가노이드 배양용 배지 조성물과 신경근 오가노이드의 제조방법. Applicant: 애니머스큐어 주식회사. The sequence listing filed with the application follows.

SEQUENCE LISTING (22 sequences)

SEQ ID NO: 1 - DNA, 20 bp, synthetic construct
  source 1..20: mol_type = other DNA
ggcatgatgggaatctccgt

SEQ ID NO: 2 - DNA, 21 bp, synthetic construct
  source 1..21: mol_type = other DNA
aggtgccaagtctgaactcac

SEQ ID NO: 3 - DNA, 22 bp, synthetic construct
  source 1..22: mol_type = other DNA
gtggctcagaacagcagcatca

SEQ ID NO: 4 - DNA, 22 bp, synthetic construct
  source 1..22: mol_type = other DNA
cctcactgagacggcggaaatt

SEQ ID NO: 5 - DNA, 22 bp, synthetic construct
  source 1..22: mol_type = other DNA
ccgaggtgaaaagtgccatcga

SEQ ID NO: 6 - DNA, 22 bp, synthetic construct
  source 1..22: mol_type = other DNA
tccgaggagtatgtggtccatc

SEQ ID NO: 7 - DNA, 22 bp, synthetic construct
  source 1..22: mol_type = other DNA
gtctcctctgacttcaacagcg

SEQ ID NO: 8 - DNA, 22 bp, synthetic construct
  source 1..22: mol_type = other DNA
accaccctgttgctgtagccaa

SEQ ID NO: 9 - DNA, 20 bp, synthetic construct
  source 1..20: mol_type = other DNA
cacctggatgatgctctccg

SEQ ID NO: 10 - DNA, 20 bp, synthetic construct
  source 1..20: mol_type = other DNA
tgatcaggctggtgttctgg

SEQ ID NO: 11 - DNA, 20 bp, synthetic construct
  source 1..20: mol_type = other DNA
agcaatagtgcagagcaggg

SEQ ID NO: 12 - DNA, 20 bp, synthetic construct
  source 1..20: mol_type = other DNA
agaggcccgagtaggtgtag

SEQ ID NO: 13 - DNA, 20 bp, synthetic construct
  source 1..20: mol_type = other DNA
cttgagtagcccaggcacag

SEQ ID NO: 14 - DNA, 20 bp, synthetic construct
  source 1..20: mol_type = other DNA
cgagacacgatcttggcctt

SEQ ID NO: 15 - DNA, 22 bp, synthetic construct
  source 1..22: mol_type = other DNA
atgcacgacctcaacatcgcca

SEQ ID NO: 16 - DNA, 22 bp, synthetic construct
  source 1..22: mol_type = other DNA
accagtcgcttcatctcctcca

SEQ ID NO: 17 - DNA, 22 bp, synthetic construct
  source 1..22: mol_type = other DNA
acaaagcacatgctgcccagtg

SEQ ID NO: 18 - DNA, 22 bp, synthetic construct
  source 1..22: mol_type = other DNA
ttccacgatggctttgcggttc

SEQ ID NO: 19 - DNA, 20 bp, synthetic construct
  source 1..20: mol_type = other DNA
ccaaaaagctgaccccttta

SEQ ID NO: 20 - DNA, 20 bp, synthetic construct
  source 1..20: mol_type = other DNA
gctccggtgttttcttcatc

SEQ ID NO: 21 - DNA, 20 bp, synthetic construct
  source 1..20: mol_type = other DNA
agtgatgagcatggcatcga

SEQ ID NO: 22 - DNA, 20 bp, synthetic construct
  source 1..20: mol_type = other DNA
aggcagtcgcagttttcaca